European Patent Specification EP 3 821 017 B1, published October 25, 2023. Title: A cell surface tag exchange (CSTE) system for tracing and manipulation of cells during recombinase mediated cassette exchange integration of nucleic acid sequences to engineered receiver cells. Applicant: Genovie AB. The sequence listing filed with the application follows.

SEQUENCE LISTING (23 sequences)

SEQ ID NO: 1 - DNA, 5837 bp, Artificial sequence
  Tag-exchange receiver site encoding Myc CST and RFP selection gene
gagctctactggcttctgcgccgcctctggcccactgtttccccttcccaggcaggtcctgctttctctgacctgcattctctcccctgggcctgtgccgctttctgtctgcagcttgtggcctgggtcacctctacggctggcccagatccttccctgccgcctccttcaggttccgtcttcctccactccctcttccccttgctctctgctgtgttgctgcccaaggatgctctttccggagcacttccttctcggcgctgcaccacgtgatgtcctctgagcggatcctccccgtgtctgggtcctctccgggcatctctcctccctcacccaaccccatgccgtcttcactcgctgggttcccttttccttctccttctggggcctgtgccatctctcgtttcttaggatggccttctccgacggatgtctcccttgcgtcccgcctccccttcttgtaggcctgcatcatcaccgtttttctggacaaccccaaagtaccccgtctccctggctttagccacctctccatcctcttgctttctttgcctggacaccccgttctcctgtggattcgggtcacctctcactcctttcatttgggcagctcccctaccccccttacctctctagtctgtgctagctcttccagccccctgtcatggcatcttccaggggtccgagagctcagctagtcttcttcctccaacccgggcccctatgtccacttcaggacagcatgtttgctgcctccagggatcctgtgtccccgagctgggaccaccttatattcccagggccggttaatgtggctctggttctgggtacttttatctgtcccctccaccgggtggctccggtgcccgtcagtgggcagagcgcacatcgcccacagtccccgagaagttggggggaggggtcggcaattgaaccggtgcctagagaaggtggcgcggggtaaactgggaaagtgatgtcgtgtactggctccgcctttttcccgagggtgggggagaaccgtatataagtgcagtagtcgccgtgaacgttctttttcgcaacgggtttgccgccagaacacaggtaagtgccgtgtgtggttcccgcgggcctggcctctttacgggttatggcccttgcgtgccttgaattacttccactggctgcagtacgtgattcttgatcccgagcttcgggttggaagtgggtgggagagttcgaggccttgcgcttaaggagccccttcgcctcgtgcttgagttgaggcctggcctgggcgctggggccgccgcgtgcgaatctggtggcaccttcgcgcctgtctcgctgctttcgataagtctctagccatttaaaatttttgatgacctgctgcgacgctttttttctggcaagatagtcttgtaaatgcgggccaagatctgcacactggtatttcggtttttggggccgcgggcggcgacggggcccgtgcgtcccagcgcacatgttcggcgaggcggggcctgcgagcgcggccaccgagaatcggacgggggtagtctcaagctggccggcctgctctggtgcctggcctcgcgccgccgtgtatcgccccgccctgggcggcaaggctggcccggtcggcaccagttgcgtgagcggaaagatggccgcttcccggccctgctgcagggagctcaaaatggaggacgcggcgctcgggagagcgggcgggtgagtcacccacacaaaggaaaagggcctttccgtcctcagccgtcgcttcatgtgactccacggagtaccgggcgccgtccaggcacctcgattagttctcgagcttttggagtacgtcgtctttaggttggggggaggggttttatgcgatggagtttccccacactgagtgggtggagactgaagttaggccagcttggcacttgatgtaattctccttggaatttgccctttttgagtttggatcttggttcattctcaagcctcagacagtggttcaaagtttttttcttccatttcaggtgtcgtgactgcttaagcttggtaccgccaccatggccaagggcttctacatcagcaagagcctgggcatcctgggaatcctgctgggagtggctgctgtgtgcaccatcatcgctctgagcgtggtgtacagccaggagggaggtcctggatccggaacaggtggctctggcactggaggatcaggtccaggtggatctatggtgaagcagatcgagagcaagactgctttccaggaagccttggacgctgcaggtgataagcttgtagtagttgacttctcagcaacgtggtctggaccttccaagatgatcaagcctttcttccattccctctctgagaagtattccaacgtgatattccttgaagtagatgtggatgactctcaggatgttgcttcagagtgtgaagtcaaatccatgccaacattccagttcttcaagaagggacagaaggtgggtgaattttctggagccaataaggagaagcttgaagccaccattaacgagttggtaggtaagtggctggggccagagactggctcttgaagttcctattccgaagttcctattctctagaaagtataggaacttcctggctcagaaaaagggccctgacaactcttttcatcttctaggcggttcctctacatccggtggatctggatctggagaacaaaagctcatctctgaggaggaccttggggagcagaagctaatcagtgaagaagacctcggagagcagaaattgattagcgaggaggatctttaaagacgctagcacctgatcctgatcataatcaagccatatcacatctgtagaggtttacttgctttaaaaaacctccacacctccccctgaacctgaaacataaaatgaatgcaattgttgttgttaacttgtttattgcagcttataatggttacaaataaagcaatagcatcacaaatttcacaaataaagcatttttttcactgcattctagttgtggtttgtccaaactcatcaatgtatcttatcatgtctggatctgctgaagagcgctgatcagctcttcaccatagagcccaccgcatccccagcatgcctgctattgtcttcccaatcctcccccttgctgtcctgccccaccccaccccccagaatagaatgacacctactcagacaatgcgatgcaatttcctcattttattaggaaaggacagtgggagtggcaccttccagggtcaaggaaggcacgggggaggggcaaacaacagatggctggcaactagaaggcacagtcgggtgctagctcatctgtggcccagcttgctaggcaggtcgcagtacttggccacggccatctcgtgctgttccacgtaggtttctttgtcggcctctttgatccgttccagccggtggtccacgaagtggaagccgggcatcttcaggttcttggcgggcttcttgcttctgtaggtggtcttgaaggagcagtgcaggtagcctccgcccacgagtttcagggccatctgagaatggcctctcaggccgccatcggcagggtacagcatctcggtgttggcctcccagcctctggttttcttctgcatcacggggccgttgctggggaagttcacgccgttaatcttcacgttgtagatgatgcagccgttctggaagctggtatcctgggtggcggtcagcactccgccgtcctcgtatgtggtgatccgctcccaggtgaagccctcggggaagctctgcttgaagaaatcggggatgccctgggtgtggttgatgaaggccttgctgccgtacataaagctggtggccaggatatcaaaggcgaagggcagagggccgccttccaccaccttgatcttcatggtctgggtgccctcgtaaggcttgccctcgccctcgctggtgcacttgaagtggtggttgttcacggtgccttccatgtacagcttcatgtgcatgttttctttgatcagctcgctcatggtggctacggaagttcctattccgaagttcctattcttcaaatagtataggaacttccggtaccagtcacgacacctgaaatggaagaaaaaaactttgaaccactgtctgaggcttgagaatgaaccaagatccaaactcaaaaagggcaaattccaaggagaattacatcaagtgccaagctggcctaacttcagtctccacccactcagtgtggggaaactccatcgcataaaacccctccccccaacctaaagacgacgtactccaaaagctcgagaactaatcgaggtgcctggacggcgcccggtactccgtggagtcacatgaagcgacggctgaggacggaaaggcccttttcctttgtgtgggtgactcacccgcccgctctcccgagcgccgcgtcctccattttgagctccctgcagcagggccgggaagcggccatctttccgctcacgcaactggtgccgaccgggccagccttgccgcccagggcggggcgatacacggcggcgcgaggccaggcaccagagcaggccggccagcttgagactacccccgtccgattctcggtggccgcgctcgcaggccccgcctcgccgaacatgtgcgctgggacgcacgggccccgtcgccgcccgcggccccaaaaaccgaaataccagtgtgcagatcttggcccgcatttacaagactatcttgccagaaaaaaagcgtcgcagcaggtcatcaaaaattttaaatggctagagacttatcgaaagcagcgagacaggcgcgaaggtgccaccagattcgcacgcggcggccccagcgcccaggccaggcctcaactcaagcacgaggcgaaggggctccttaagcgcaaggcctcgaactctcccacccacttccaacccgaagctcgggatcaagaatcacgtactgcagccagtggaagtaattcaaggcacgcaagggccataacccgtaaagaggccaggcccgcgggaaccacacacggcacttacctgtgttctggcggcaaacccgttgcgaaaaagaacgttcacggcgactactgcacttatatacggttctcccccaccctcgggaaaaaggcggagccagtacacgacatcactttcccagtttaccccgcgccaccttctctaggcaccggttcaattgccgacccctccccccaacttctcggggactgtgggcgatgtgcgctctgcccactgacgggcaccggagccaccggatcaggatcaggattggtgacagaaaagccccatccttaggcctcctccttcctagtctcctgatattgggtctaacccccacctcctgttaggcagattccttatctggtgacacacccccatttcctggagccatctctctccttgccagaacctctaaggtttgcttacgatggagccagagaggatcctgggagggagagcttggcagggggtgggagggaagggggggatgcgtgacctgcccggttctcagtggccaccctgcgctaccctctcccagaacctgagctgctctgacgcggctgtctggtgcgtttcactgatcctggtgctgcagcttccttacacttcccaagaggagaagcagtttggaaaaacaaaatcagaataagttggtcctgagttctaactttggctcttcacctttctagtccccaatttatattgttcctccgtgcgtcagttttacctgtgagataaggccagtagccagccccgtcctggcagggctgtggtgaggaggggggtgtccgtgtggaaaactccctttgtgagaatggtgcgtcc

SEQ ID NO: 2 - DNA, 1332 bp, Artificial sequence
  Flippase
atggcccccaagaaaaagcggaaagtgggcatccacggcgtgccagctgcaggcggctctatgagccagttcgacatcctgtgcaagaccccacctaaggtgctcgtgcggcagttcgtggaaagattcgagaggcctagcggcgagaagatcgcctcttgtgctgccgagctgacctacctgtgctggatgatcacccacaacggcaccgccatcaagcgggccaccttcatgagctacaataccatcatcagcaacagcctgagcttcgacatcgtgaacaagagcctgcagttcaagtacaagacccagaaggccaccatcctggaagccagcctgaagaaactgatccccgcctgggagtttaccatcatcccatacaatggccagaaacatcagagcgacattaccgatatcgtgtccagcctccagctgcagttcgagagtagcgaagaagccgacaagggcaacagccacagcaagaagatgctgaaggccctgctgagcgagggcgagagcatctgggagatcacagagaagatcctgaacagcttcgagtacaccagccggttcaccaagaccaagaccctgtaccagttcctgttcctggccacctttatcaactgcggccggttctccgacatcaagaacgtggaccccaagagcttcaagctggtgcagaacaagtacctgggcgtgatcattcagtgcctcgtgaccgagacaaagaccagcgtgtcccggcacatctactttttcagcgccagaggccggatcgaccccctggtgtacctggacgagttcctgagaaacagcgagcccgtgctgaagagagtgaaccggaccggcaacagcagctccaacaagcaggaataccagctgctgaaggacaacctcgtgcggtcctacaacaaggccctgaagaaaaacgccccctaccccatcttcgccattaagaacggccccaagtcccacatcggccggcacctgatgaccagctttctgagcatgaagggcctgacagagctgaccaacgtcgtgggcaattggagcgacaagagggcctctgccgtggccagaaccacctacacccaccagatcacagccatccccgaccactacttcgccctggtgtctcggtactacgcctacgaccccatcagcaaagagatgatcgccctgaaggacgagacaaaccccatcgaggaatggcagcacatcgagcagctgaagggcagcgccgagggcagcatcagataccctgcctggaacggcatcatctcccaggaagtgctggactacctgagcagctacatcaaccggcggatctga

SEQ ID NO: 3 - DNA, 1791 bp, Artificial sequence
  TEDV encoding SBP CST and P-gene_RSV1 GOI
gaagttcctattccgaagttcctattctctagaaagtataggaacttcctggctcagaaaaagggccctgacaactcttttcatcttctaggcggttcctctacatccggtggatctggatctgggcatgtggttgaggggcttgctggcgaactagagcaattgcgagcccgcctcgaacaccatcctcaaggtcaataaagactcgagcacctgatcctgatcataatcaagccatatcacatctgtagaggtttacttgctttaaaaaacctccacacctccccctgaacctgaaacataaaatgaatgcaattgttgttgttaacttgtttattgcagcttataatggttacaaataaagcaatagcatcacaaatttcacaaataaagcatttttttcactgcattctagttgtggtttgtccaaactcatcaatgtatcttatcatgtctggatctgctgaagagcgctgatcagctcttcaccatagagcccaccgcatccccagcatgcctgctattgtcttcccaatcctcccccttgctgtcctgccccaccccaccccccagaatagaatgacacctactcagacaatgcgatgcaatttcctcattttattaggaaaggacagtgggagtggcaccttccagggtcaaggaaggcacgggggaggggcaaacaacagatggctggcaactagaaggcacagtcgggtgctagcgaagaccgagcggtggatccgtatggtgacaagacgactagtgtgaacgactagaaagagaacccggcacatctgtcgagaggtacgaccgtgcactaagcttcgcaaggtcagtggagctatcgagtgtaggatggttcaagtctgccaatggagctacagaagtcgaagccgtccagatctggactatagtcacttatcgtcatcgtccttataatcaatatcgtggtctttataatctccatcatgatccttgtaatccccggggaaatcttccaggctcaggtcgttgtcgctgtcgttgccttccagcaggttgttcagcttctcagaggtagggttcagagacacttcgtcggaggtgtccttggccatcttctcggattcctcgtttctcagccgggccatagcttccagccgatcgttggtcatcagggcctctgtccggatcttctcgatcatctcttcccgcagtccgaccatggcatctctgatgccatctctggcagatgtaggtccggcagatgccaccaccagtgtgtgcagcatgcccaggatctcagacagcttctcgtcgatccggtccagtctggcggtgatgttgtcgttggtctggtcgttgatttcctcgtagctgtagctgctctcttcctcgttgttgtcgaatgtctcgattgtctctttgtacagcttgctgaaggggttgtcgctaggtgtggggtcctctttgaaggacaccaggggctttctctggtagttgggcttgttgccggcggtgtcgtctgtctcgttggtggggttgatgatggtgctgttgctggtgatggggctctctttggtcacttcgatgtcgatgctgttcacgctgatgatgctgtccttcttcttggggtccttggggctcgtgaacttgcccttgatggattccagaaacttggtggcccgattgttggcgtcctcgccgtggaactcaggggcgaacttttccatggtggcggtattgtcttcggtaccgcacgaagttcctattcggaagttcctattcttcaaatagtataggaacttc

SEQ ID NO: 4 - DNA, 2241 bp, Artificial sequence
  TEDV encoding SBP CST and N-gene_RSV1 GOI
gaagttcctattccgaagttcctattctctagaaagtataggaacttcctggctcagaaaaagggccctgacaactcttttcatcttctaggcggttcctctacatccggtggatctggatctgggcatgtggttgaggggcttgctggcgaactagagcaattgcgagcccgcctcgaacaccatcctcaaggtcaataaagactcgagcacctgatcctgatcataatcaagccatatcacatctgtagaggtttacttgctttaaaaaacctccacacctccccctgaacctgaaacataaaatgaatgcaattgttgttgttaacttgtttattgcagcttataatggttacaaataaagcaatagcatcacaaatttcacaaataaagcatttttttcactgcattctagttgtggtttgtccaaactcatcaatgtatcttatcatgtctggatctgctgaagagcgctgatcagctcttcaccatagagcccaccgcatccccagcatgcctgctattgtcttcccaatcctcccccttgctgtcctgccccaccccaccccccagaatagaatgacacctactcagacaatgcgatgcaatttcctcattttattaggaaaggacagtgggagtggcaccttccagggtcaaggaaggcacgggggaggggcaaacaacagatggctggcaactagaaggcacagtcgggtgctagcgaagaccgagcggtggatccgtatggtgacaagacgactagtgtgaacgactagggagagaacccggcacatctgtcgagaggtacgaccgtgcactaagcttcgcaaggtcagtggagctatcgagtgtaggatggttcaagtctgccaatggagctacagaagtcgaagccgtccagatctggactatagtcacttatcgtcatcgtccttataatcaatatcgtggtctttataatctccatcatgatccttgtaatccccgggcagttccacgtcgttgtccttagggttcagctggtgcttgatggcttccagttcctcggcggtcagatccagcacgctgtagttgatcacgccgttttctttcagctgctcggcataggccttggcggcatcgtacaggtcctggtttctaggggtgcctctgtactcgcccatgattcccagtccggcggcatttcccagcaccacagagctgaagtgtgggaactgtgtcaggctcagcagagaggccttggggttgttcaggatgtggtaaaagccggcctctccgccaagcttctgggcgtactcgtacacttccaccacctgttccatttcggcctgcacagaggcgtggcccagcatgatgttcttcacgctcttggccagcactccccatctcagcatcacttgtccggcgccataggcattcatgaacaggccggcgaagatgccttccacccgagagccgcctcttgtgctgctctgggcgattccgaagtgcacgaacacgtcgatgaagtgagggtacttctcgaacacctcgtagaagctgttggcaatatccttaggcagcaggcccttgtaccgcttcatctcgttcttcagcacgttgttggctctccgaatcacagcggtcaggccagaccgatcgccagcggccagtttggtgatgaccagagcggcgatacacaggatgatcatgccgcaatcagggctgtcgtgtctgtactcaggggcgacttcgcccatctctttcagcattttcttgtaggacttccggctctcgatctcgatgttgatctggatctctgtggtcaggctggccagggtcagcacctcgaacttcatttctttgccgttgatgtcctgccggtgtgtggtcacgtccacgccattggccttcacgtggtagccggcatctctcaggatcttgatggtgtcctctctgcccagtctgctcatggcgtacagcattccgatcacgcctgtgaacttgtggttggcgtcctcggtgatcagcagcatgccgcacagcttgttgatgtgcttctgcacgtcgtagttaggggtgtcgatgctgtcgccggtgcttctctggatggtgtacttgctgctgctcagcagctggtccttgttcagggtgtcgttcagcttcactttgctcagggccatggtggcggtattgtcttcggtaccgcacgaagttcctattcggaagttcctattcttcaaatagtataggaacttc

SEQ ID NO: 5 - DNA, 1649 bp, Artificial sequence
  M2-long-gene_RSV1
gaagttcctattccgaagttcctattctctagaaagtataggaacttcctggctcagaaaaagggccctgacaactcttttcatcttctaggcggttcctctacatccggtggatctggatctgggcatgtggttgaggggcttgctggcgaactagagcaattgcgagcccgcctcgaacaccatcctcaaggtcaataaagactcgagcacctgatcctgatcataatcaagccatatcacatctgtagaggtttacttgctttaaaaaacctccacacctccccctgaacctgaaacataaaatgaatgcaattgttgttgttaacttgtttattgcagcttataatggttacaaataaagcaatagcatcacaaatttcacaaataaagcatttttttcactgcattctagttgtggtttgtccaaactcatcaatgtatcttatcatgtctggatctgctgaagagcgctgatcagctcttcaccatagagcccaccgcatccccagcatgcctgctattgtcttcccaatcctcccccttgctgtcctgccccaccccaccccccagaatagaatgacacctactcagacaatgcgatgcaatttcctcattttattaggaaaggacagtgggagtggcaccttccagggtcaaggaaggcacgggggaggggcaaacaacagatggctggcaactagaaggcacagtcgggtgctagcgaagaccgagcggtggatccgtatggtgacaagacgactagtgtgaacgacctgttagagaacccggcacatctgtcgagaggtacgaccgtgcactaagcttcgcaaggtcagtggagctatcgagtgtaggatggttcaagtctgccaatggagctacagaagtcgaagccgtccagatctggactatagtcacttatcgtcatcgtccttataatcaatatcgtggtctttataatctccatcatgatccttgtaatccccgggggtggtatcgttgttcttggcgtggtcgttggtgtcgttgacggtgctctctttgggattgttgatggtgatgctcttgtggatgtccagggtgttcttgatggttttcttcagcacgtcggcaggcagccgcttcagcagatggatggtctgcttgttgttcttccggttgctctcgatgtagctgatcacggtgttgtacacccggatcttggggctgttaggttcctcgttgtcccgcagcttcttgatgtcgtcgctgttcagctctgtcagcagcttgctcatggccacgcaggcgctctgcttggtgatgttgttgatgctgccgatatagctttccagcacgcccacaacgcccagggcatattcctcggttctatccagttcggcggctccgctgatctcgctcagggtgtcgatgctcttatccatggacttcaggattctgttcagcatgaagttctgccgcacgagcagagcgtgaggaggccactcgaagtagttgtggctgaagtggcatctcttgccgttcaggcagtggcctctgatctcgaacttgcaggggttccgtctgctcatggtggcggtattgtcttcggtaccgcacgaagttcctattcggaagttcctattcttcaaatagtataggaactt

SEQ ID NO: 6 - DNA, 4542 bp, Artificial sequence
  CMVpro-Flp-sv40pA-V2 vector V4.I.8
ctaaattgtaagcgttaatattttgttaaaattcgcgttaaatttttgttaaatcagctcattttttaaccaataggccgaaatcggcaaaatcccttataaatcaaaagaatagaccgagatagggttgagtggccgctacagggcgctcccattcgccattcaggctgcgcaactgttgggaagggcgtttcggtgcgggcctcttcgctattacgccagctggcgaaagggggatgtgctgcaaggcgattaagttgggtaacgccagggttttcccagtcacgacgttgtaaaacgacggccagtgagcgcgacgtaatacgactcactatagggcgaattggcggaaggccgtcaaggccgcatgaattcgctaccggtatagtaatcaattacggggtcattagttcatagcccatatatggagttccgcgttacataacttacggtaaatggcccgcctggctgaccgcccaacgacccccgcccattgacgtcaataatgacgtatgttcccatagtaacgccaatagggactttccattgacgtcaatgggtggagtatttacggtaaactgcccacttggcagtacatcaagtgtatcatatgccaagtacgccccctattgacgtcaatgacggtaaatggcccgcctggcattatgcccagtacatgaccttatgggactttcctacttggcagtacatctacgtattagtcatcgctattaccatggtgatgcggttttggcagtacatcaatgggcgtggatagcggtttgactcacggggatttccaagtctccaccccattgacgtcaatgggagtttgttttggcaccaaaatcaacgggactttccaaaatgtcgtaacaactccgccccattgacgcaaatgggcggtaggcgtgtacggtgggaggtctatataagcagagctggtttagtgaaccgtcagatcaggtaccatggcccccaagaaaaagcggaaagtgggcatccacggcgtgccagctgcaggcggctctatgagccagttcgacatcctgtgcaagaccccacctaaggtgctcgtgcggcagttcgtggaaagattcgagaggcctagcggcgagaagatcgcctcttgtgctgccgagctgacctacctgtgctggatgatcacccacaacggcaccgccatcaagcgggccaccttcatgagctacaataccatcatcagcaacagcctgagcttcgacatcgtgaacaagagcctgcagttcaagtacaagacccagaaggccaccatcctggaagccagcctgaagaaactgatccccgcctgggagtttaccatcatcccatacaatggccagaaacatcagagcgacattaccgatatcgtgtccagcctccagctgcagttcgagagtagcgaagaagccgacaagggcaacagccacagcaagaagatgctgaaggccctgctgagcgagggcgagagcatctgggagatcacagagaagatcctgaacagcttcgagtacaccagccggttcaccaagaccaagaccctgtaccagttcctgttcctggccacctttatcaactgcggccggttctccgacatcaagaacgtggaccccaagagcttcaagctggtgcagaacaagtacctgggcgtgatcattcagtgcctcgtgaccgagacaaagaccagcgtgtcccggcacatctactttttcagcgccagaggccggatcgaccccctggtgtacctggacgagttcctgagaaacagcgagcccgtgctgaagagagtgaaccggaccggcaacagcagctccaacaagcaggaataccagctgctgaaggacaacctcgtgcggtcctacaacaaggccctgaagaaaaacgccccctaccccatcttcgccattaagaacggccccaagtcccacatcggccggcacctgatgaccagctttctgagcatgaagggcctgacagagctgaccaacgtcgtgggcaattggagcgacaagagggcctctgccgtggccagaaccacctacacccaccagatcacagccatccccgaccactacttcgccctggtgtctcggtactacgcctacgaccccatcagcaaagagatgatcgccctgaaggacgagacaaaccccatcgaggaatggcagcacatcgagcagctgaagggcagcgccgagggcagcatcagataccctgcctggaacggcatcatctcccaggaagtgctggactacctgagcagctacatcaaccggcggatctgatctagacctgatcataatcaagccatatcacatctgtagaggtttacttgctttaaaaaacctccacacctccccctgaacctgaaacataaaatgaatgcaattgttgttgttaacttgtttattgcagcttataatggttacaaataaagcaatagcatcacaaatttcacaaataaagcatttttttcactgcattctagttgtggtttgtccaaactcatcaatgtatcttatcatgtctggatctgcggatccaatctcgagctgggcctcatgggccttccgctcactgcccgctttccagtcgggaaacctgtcgtgccagctgcattaacatggtcatagctgtttccttgcgtattgggcgctctccgcttcctcgctcactgactcgctgcgctcggtcgttcgggtaaagcctggggtgcctaatgagcaaaaggccagcaaaaggccaggaaccgtaaaaaggccgcgttgctggcgtttttccataggctccgcccccctgacgagcatcacaaaaatcgacgctcaagtcagaggtggcgaaacccgacaggactataaagataccaggcgtttccccctggaagctccctcgtgcgctctcctgttccgaccctgccgcttaccggatacctgtccgcctttctcccttcgggaagcgtggcgctttctcatagctcacgctgtaggtatctcagttcggtgtaggtcgttcgctccaagctgggctgtgtgcacgaaccccccgttcagcccgaccgctgcgccttatccggtaactatcgtcttgagtccaacccggtaagacacgacttatcgccactggcagcagccactggtaacaggattagcagagcgaggtatgtaggcggtgctacagagttcttgaagtggtggcctaactacggctacactagaagaacagtatttggtatctgcgctctgctgaagccagttaccttcggaaaaagagttggtagctcttgatccggcaaacaaaccaccgctggtagcggtggtttttttgtttgcaagcagcagattacgcgcagaaaaaaaggatctcaagaagatcctttgatcttttctacggggtctgacgctcagtggaacgaaaactcacgttaagggattttggtcatgagattatcaaaaaggatcttcacctagatccttttaaattaaaaatgaagttttaaatcaatctaaagtatatatgagtaaacttggtctgacagttaccaatgcttaatcagtgaggcacctatctcagcgatctgtctatttcgttcatccatagttgcctgactccccgtcgtgtagataactacgatacgggagggcttaccatctggccccagtgctgcaatgataccgcgagaaccacgctcaccggctccagatttatcagcaataaaccagccagccggaagggccgagcgcagaagtggtcctgcaactttatccgcctccatccagtctattaattgttgccgggaagctagagtaagtagttcgccagttaatagtttgcgcaacgttgttgccattgctacaggcatcgtggtgtcacgctcgtcgtttggtatggcttcattcagctccggttcccaacgatcaaggcgagttacatgatcccccatgttgtgcaaaaaagcggttagctccttcggtcctccgatcgttgtcagaagtaagttggccgcagtgttatcactcatggttatggcagcactgcataattctcttactgtcatgccatccgtaagatgcttttctgtgactggtgagtactcaaccaagtcattctgagaatagtgtatgcggcgaccgagttgctcttgcccggcgtcaatacgggataataccgcgccacatagcagaactttaaaagtgctcatcattggaaaacgttcttcggggcgaaaactctcaaggatcttaccgctgttgagatccagttcgatgtaacccactcgtgcacccaactgatcttcagcatcttttactttcaccagcgtttctgggtgagcaaaaacaggaaggcaaaatgccgcaaaaaagggaataagggcgacacggaaatgttgaatactcatactcttcctttttcaatattattgaagcatttatcagggttattgtctcatgagcggatacatatttgaatgtatttagaaaaataaacaaataggggttccgcgcacatttccccgaaaagtgccac

SEQ ID NO: 7 - DNA, 10428 bp, Artificial sequence
  SpCas9-2A-GFP vector V1.A.8
gacggatcgggagatctcccgatcccctatggtgcactctcagtacaatctgctctgatgccgcatagttaagccagtatctgctccctgcttgtgtgttggaggtcgctgagtagtgcgcgagcaaaatttaagctacaacaaggcaaggcttgaccgacaattgcatgaagaatctgcttagggttaggcgttttgcgctgcttcgcgatgtacgggccagatatacgcgttgacattgattattgactagttattaatagtaatcaattacggggtcattagttcatagcccatatatggagttccgcgttacataacttacggtaaatggcccgcctggctgaccgcccaacgacccccgcccattgacgtcaataatgacgtatgttcccatagtaacgccaatagggactttccattgacgtcaatgggtggagtatttacggtaaactgcccacttggcagtacatcaagtgtatcatatgccaagtacgccccctattgacgtcaatgacggtaaatggcccgcctggcattatgcccagtacatgaccttatgggactttcctacttggcagtacatctacgtattagtcatcgctattaccatggtgatgcggttttggcagtacatcaatgggcgtggatagcggtttgactcacggggatttccaagtctccaccccattgacgtcaatgggagtttgttttggcaccaaaatcaacgggactttccaaaatgtcgtaacaactccgccccattgacgcaaatgggcggtaggcgtgtacggtgggaggtctatataagcagagctctctggctaactagagaacccactgcttactggcttatcgaaattaatacgactcactatagggagacccaagctggctagcgtttaaacttaagcttggtaccgccaccatggactataaggaccacgacggagactacaaggatcatgatattgattacaaagacgatgacgataagatggccccaaagaagaagcggaaggtcggtatccacggagtcccagcagccgacaagaagtacagcatcggcctggacatcggcaccaactctgtgggctgggccgtgatcaccgacgagtacaaggtgcccagcaagaaattcaaggtgctgggcaacaccgaccggcacagcatcaagaagaacctgatcggagccctgctgttcgacagcggcgaaacagccgaggccacccggctgaagagaaccgccagaagaagatacaccagacggaagaaccggatctgctatctgcaagagatcttcagcaacgagatggccaaggtggacgacagcttcttccacagactggaagagtccttcctggtggaagaggataagaagcacgagcggcaccccatcttcggcaacatcgtggacgaggtggcctaccacgagaagtaccccaccatctaccacctgagaaagaaactggtggacagcaccgacaaggccgacctgcggctgatctatctggccctggcccacatgatcaagttccggggccacttcctgatcgagggcgacctgaaccccgacaacagcgacgtggacaagctgttcatccagctggtgcagacctacaaccagctgttcgaggaaaaccccatcaacgccagcggcgtggacgccaaggccatcctgtctgccagactgagcaagagcagacggctggaaaatctgatcgcccagctgcccggcgagaagaagaatggcctgttcggaaacctgattgccctgagcctgggcctgacccccaacttcaagagcaacttcgacctggccgaggatgccaaactgcagctgagcaaggacacctacgacgacgacctggacaacctgctggcccagatcggcgaccagtacgccgacctgtttctggccgccaagaacctgtccgacgccatcctgctgagcgacatcctgagagtgaacaccgagatcaccaaggcccccctgagcgcctctatgatcaagagatacgacgagcaccaccaggacctgaccctgctgaaagctctcgtgcggcagcagctgcctgagaagtacaaagagattttcttcgaccagagcaagaacggctacgccggctacattgacggcggagccagccaggaagagttctacaagttcatcaagcccatcctggaaaagatggacggcaccgaggaactgctcgtgaagctgaacagagaggacctgctgcggaagcagcggaccttcgacaacggcagcatcccccaccagatccacctgggagagctgcacgccattctgcggcggcaggaagatttttacccattcctgaaggacaaccgggaaaagatcgagaagatcctgaccttccgcatcccctactacgtgggccctctggccaggggaaacagcagattcgcctggatgaccagaaagagcgaggaaaccatcaccccctggaacttcgaggaagtggtggacaagggcgcttccgcccagagcttcatcgagcggatgaccaacttcgataagaacctgcccaacgagaaggtgctgcccaagcacagcctgctgtacgagtacttcaccgtgtataacgagctgaccaaagtgaaatacgtgaccgagggaatgagaaagcccgccttcctgagcggcgagcagaaaaaggccatcgtggacctgctgttcaagaccaaccggaaagtgaccgtgaagcagctgaaagaggactacttcaagaaaatcgagtgcttcgactccgtggaaatctccggcgtggaagatcggttcaacgcctccctgggcacataccacgatctgctgaaaattatcaaggacaaggacttcctggacaatgaggaaaacgaggacattctggaagatatcgtgctgaccctgacactgtttgaggacagagagatgatcgaggaacggctgaaaacctatgcccacctgttcgacgacaaagtgatgaagcagctgaagcggcggagatacaccggctggggcaggctgagccggaagctgatcaacggcatccgggacaagcagtccggcaagacaatcctggatttcctgaagtccgacggcttcgccaacagaaacttcatgcagctgatccacgacgacagcctgacctttaaagaggacatccagaaagcccaggtgtccggccagggcgatagcctgcacgagcacattgccaatctggccggcagccccgccattaagaagggcatcctgcagacagtgaaggtggtggacgagctcgtgaaagtgatgggccggcacaagcccgagaacatcgtgatcgaaatggccagagagaaccagaccacccagaagggacagaagaacagccgcgagagaatgaagcggatcgaagagggcatcaaagagctgggcagccagatcctgaaagaacaccccgtggaaaacacccagctgcagaacgagaagctgtacctgtactacctgcagaatgggcgggatatgtacgtggaccaggaactggacatcaaccggctgtccgactacgatgtggaccatatcgtgcctcagagctttctgaaggacgactccatcgacaacaaggtgctgaccagaagcgacaagaaccggggcaagagcgacaacgtgccctccgaagaggtcgtgaagaagatgaagaactactggcggcagctgctgaacgccaagctgattacccagagaaagttcgacaatctgaccaaggccgagagaggcggcctgagcgaactggataaggccggcttcatcaagagacagctggtggaaacccggcagatcacaaagcacgtggcacagatcctggactcccggatgaacactaagtacgacgagaatgacaagctgatccgggaagtgaaagtgatcaccctgaagtccaagctggtgtccgatttccggaaggatttccagttttacaaagtgcgcgagatcaacaactaccaccacgcccacgacgcctacctgaacgccgtcgtgggaaccgccctgatcaaaaagtaccctaagctggaaagcgagttcgtgtacggcgactacaaggtgtacgacgtgcggaagatgatcgccaagagcgagcaggaaatcggcaaggctaccgccaagtacttcttctacagcaacatcatgaactttttcaagaccgagattaccctggccaacggcgagatccggaagcggcctctgatcgagacaaacggcgaaaccggggagatcgtgtgggataagggccgggattttgccaccgtgcggaaagtgctgagcatgccccaagtgaatatcgtgaaaaagaccgaggtgcagacaggcggcttcagcaaagagtctatcctgcccaagaggaacagcgataagctgatcgccagaaagaaggactgggaccctaagaagtacggcggcttcgacagccccaccgtggcctattctgtgctggtggtggccaaagtggaaaagggcaagtccaagaaactgaagagtgtgaaagagctgctggggatcaccatcatggaaagaagcagcttcgagaagaatcccatcgactttctggaagccaagggctacaaagaagtgaaaaaggacctgatcatcaagctgcctaagtactccctgttcgagctggaaaacggccggaagagaatgctggcctctgccggcgaactgcagaagggaaacgaactggccctgccctccaaatatgtgaacttcctgtacctggccagccactatgagaagctgaagggctcccccgaggataatgagcagaaacagctgtttgtggaacagcacaagcactacctggacgagatcatcgagcagatcagcgagttctccaagagagtgatcctggccgacgctaatctggacaaagtgctgtccgcctacaacaagcaccgggataagcccatcagagagcaggccgagaatatcatccacctgtttaccctgaccaatctgggagcccctgccgccttcaagtactttgacaccaccatcgaccggaagaggtacaccagcaccaaagaggtgctggacgccaccctgatccaccagagcatcaccggcctgtacgagacacggatcgacctgtctcagctgggaggcgacaaaaggccggcggccacgaaaaaggccggccaggcaaaaaagaaaaaggaattcggcagtggagagggcagaggaagtctgctaacatgcggtgacgtcgaggagaatcctggcccagtgagcaagggcgaggagctgttcaccggggtggtgcccatcctggtcgagctggacggcgacgtaaacggccacaagttcagcgtgtccggcgagggcgagggcgatgccacctacggcaagctgaccctgaagttcatctgcaccaccggcaagctgcccgtgccctggcccaccctcgtgaccaccctgacctacggcgtgcagtgcttcagccgctaccccgaccacatgaagcagcacgacttcttcaagtccgccatgcccgaaggctacgtccaggagcgcaccatcttcttcaaggacgacggcaactacaagacccgcgccgaggtgaagttcgagggcgacaccctggtgaaccgcatcgagctgaagggcatcgacttcaaggaggacggcaacatcctggggcacaagctggagtacaactacaacagccacaacgtctatatcatggccgacaagcagaagaacggcatcaaggtgaacttcaagatccgccacaacatcgaggacggcagcgtgcagctcgccgaccactaccagcagaacacccccatcggcgacggccccgtgctgctgcccgacaaccactacctgagcacccagtccgccctgagcaaagaccccaacgagaagcgcgatcacatggtcctgctggagttcgtgaccgccgccgggatcactctcggcatggacgagctgtacaaggaattctaacgctagagggcccgtttaaacccgctgatcagcctcgactgtgccttctagttgccagccatctgttgtttgcccctcccccgtgccttccttgaccctggaaggtgccactcccactgtcctttcctaataaaatgaggaaattgcatcgcattgtctgagtaggtgtcattctattctggggggtggggtggggcaggacagcaagggggaggattgggaagacaatagcaggcatgctggggatgcggtgggctctatggcttctgaggcggaaagaaccagctggggctctagggggtatccccacgcgccctgtagcggcgcattaagcgcggcgggtgtggtggttacgcgcagcgtgaccgctacacttgccagcgccctagcgcccgctcctttcgctttcttcccttcctttctcgccacgttcgccggctttccccgtcaagctctaaatcgggggctccctttagggttccgatttagtgctttacggcacctcgaccccaaaaaacttgattagggtgatggttcacgtagtgggccatcgccctgatagacggtttttcgccctttgacgttggagtccacgttctttaatagtggactcttgttccaaactggaacaacactcaaccctatctcggtctattcttttgatttataagggattttgccgatttcggcctattggttaaaaaatgagctgatttaacaaaaatttaacgcgaattaattctgtggaatgtgtgtcagttagggtgtggaaagtccccaggctccccagcaggcagaagtatgcaaagcatgcatctcaattagtcagcaaccaggtgtggaaagtccccaggctccccagcaggcagaagtatgcaaagcatgcatctcaattagtcagcaaccatagtcccgcccctaactccgcccatcccgcccctaactccgcccagttccgcccattctccgccccatggctgactaattttttttatttatgcagaggccgaggccgcctctgcctctgagctattccagaagtagtgaggaggcttttttggaggcctaggcttttgcaaaaagctcccgggagcttgtatatccattttcggatctgatcaagagacaggatgaggatcgtttcgcatgattgaacaagatggattgcacgcaggttctccggccgcttgggtggagaggctattcggctatgactgggcacaacagacaatcggctgctctgatgccgccgtgttccggctgtcagcgcaggggcgcccggttctttttgtcaagaccgacctgtccggtgccctgaatgaactgcaggacgaggcagcgcggctatcgtggctggccacgacgggcgttccttgcgcagctgtgctcgacgttgtcactgaagcgggaagggactggctgctattgggcgaagtgccggggcaggatctcctgtcatctcaccttgctcctgccgagaaagtatccatcatggctgatgcaatgcggcggctgcatacgcttgatccggctacctgcccattcgaccaccaagcgaaacatcgcatcgagcgagcacgtactcggatggaagccggtcttgtcgatcaggatgatctggacgaagagcatcaggggctcgcgccagccgaactgttcgccaggctcaaggcgcgcatgcccgacggcgaggatctcgtcgtgacccatggcgatgcctgcttgccgaatatcatggtggaaaatggccgcttttctggattcatcgactgtggccggctgggtgtggcggaccgctatcaggacatagcgttggctacccgtgatattgctgaagagcttggcggcgaatgggctgaccgcttcctcgtgctttacggtatcgccgctcccgattcgcagcgcatcgccttctatcgccttcttgacgagttcttctgagcgggactctggggttcgaaatgaccgaccaagcgacgcccaacctgccatcacgagatttcgattccaccgccgccttctatgaaaggttgggcttcggaatcgttttccgggacgccggctggatgatcctccagcgcggggatctcatgctggagttcttcgcccaccccaacttgtttattgcagcttataatggttacaaataaagcaatagcatcacaaatttcacaaataaagcatttttttcactgcattctagttgtggtttgtccaaactcatcaatgtatcttatcatgtctgtataccgtcgacctctagctagagcttggcgtaatcatggtcatagctgtttcctgtgtgaaattgttatccgctcacaattccacacaacatacgagccggaagcataaagtgtaaagcctggggtgcctaatgagtgagctaactcacattaattgcgttgcgctcactgcccgctttccagtcgggaaacctgtcgtgccagctgcattaatgaatcggccaacgcgcggggagaggcggtttgcgtattgggcgctcttccgcttcctcgctcactgactcgctgcgctcggtcgttcggctgcggcgagcggtatcagctcactcaaaggcggtaatacggttatccacagaatcaggggataacgcaggaaagaacatgtgagcaaaaggccagcaaaaggccaggaaccgtaaaaaggccgcgttgctggcgtttttccataggctccgcccccctgacgagcatcacaaaaatcgacgctcaagtcagaggtggcgaaacccgacaggactataaagataccaggcgtttccccctggaagctccctcgtgcgctctcctgttccgaccctgccgcttaccggatacctgtccgcctttctcccttcgggaagcgtggcgctttctcatagctcacgctgtaggtatctcagttcggtgtaggtcgttcgctccaagctgggctgtgtgcacgaaccccccgttcagcccgaccgctgcgccttatccggtaactatcgtcttgagtccaacccggtaagacacgacttatcgccactggcagcagccactggtaacaggattagcagagcgaggtatgtaggcggtgctacagagttcttgaagtggtggcctaactacggctacactagaagaacagtatttggtatctgcgctctgctgaagccagttaccttcggaaaaagagttggtagctcttgatccggcaaacaaaccaccgctggtagcggtttttttgtttgcaagcagcagattacgcgcagaaaaaaaggatctcaagaagatcctttgatcttttctacggggtctgacgctcagtggaacgaaaactcacgttaagggattttggtcatgagattatcaaaaaggatcttcacctagatccttttaaattaaaaatgaagttttaaatcaatctaaagtatatatgagtaaacttggtctgacagttaccaatgcttaatcagtgaggcacctatctcagcgatctgtctatttcgttcatccatagttgcctgactccccgtcgtgtagataactacgatacgggagggcttaccatctggccccagtgctgcaatgataccgcgagacccacgctcaccggctccagatttatcagcaataaaccagccagccggaagggccgagcgcagaagtggtcctgcaactttatccgcctccatccagtctattaattgttgccgggaagctagagtaagtagttcgccagttaatagtttgcgcaacgttgttgccattgctacaggcatcgtggtgtcacgctcgtcgtttggtatggcttcattcagctccggttcccaacgatcaaggcgagttacatgatcccccatgttgtgcaaaaaagcggttagctccttcggtcctccgatcgttgtcagaagtaagttggccgcagtgttatcactcatggttatggcagcactgcataattctcttactgtcatgccatccgtaagatgcttttctgtgactggtgagtactcaaccaagtcattctgagaatagtgtatgcggcgaccgagttgctcttgcccggcgtcaatacgggataataccgcgccacatagcagaactttaaaagtgctcatcattggaaaacgttcttcggggcgaaaactctcaaggatcttaccgctgttgagatccagttcgatgtaacccactcgtgcacccaactgatcttcagcatcttttactttcaccagcgtttctgggtgagcaaaaacaggaaggcaaaatgccgcaaaaaagggaataagggcgacacggaaatgttgaatactcatactcttcctttttcaatattattgaagcatttatcagggttattgtctcatgagcggatacatatttgaatgtatttagaaaaataaacaaataggggttccgcgcacatttccccgaaaagtgccacctgacgtc

SEQ ID NO: 8 - DNA, 6071 bp, Artificial sequence
  pcDNA3.1_GFP vector V1.A.4
gacggatcgggagatctcccgatcccctatggtgcactctcagtacaatctgctctgatgccgcatagttaagccagtatctgctccctgcttgtgtgttggaggtcgctgagtagtgcgcgagcaaaatttaagctacaacaaggcaaggcttgaccgacaattgcatgaagaatctgcttagggttaggcgttttgcgctgcttcgcgatgtacgggccagatatacgcgttgacattgattattgactagttattaatagtaatcaattacggggtcattagttcatagcccatatatggagttccgcgttacataacttacggtaaatggcccgcctggctgaccgcccaacgacccccgcccattgacgtcaataatgacgtatgttcccatagtaacgccaatagggactttccattgacgtcaatgggtggagtatttacggtaaactgcccacttggcagtacatcaagtgtatcatatgccaagtacgccccctattgacgtcaatgacggtaaatggcccgcctggcattatgcccagtacatgaccttatgggactttcctacttggcagtacatctacgtattagtcatcgctattaccatggtgatgcggttttggcagtacatcaatgggcgtggatagcggtttgactcacggggatttccaagtctccaccccattgacgtcaatgggagtttgttttggcaccaaaatcaacgggactttccaaaatgtcgtaacaactccgccccattgacgcaaatgggcggtaggcgtgtacggtgggaggtctatataagcagagctctctggctaactagagaacccactgcttactggcttatcgaaattaatacgactcactatagggagacccaagctggctagcgtttaaacttaagcttggtaccgccaccatggaatccgatgagtctggcctgcccgccatggaaatcgagtgcagaatcaccggcaccctgaacggcgtggaatttgagctcgtgggcggaggcgagggcacacctgaacagggcagaatgaccaacaagatgaagtccaccaagggggccctgaccttcagcccctacctgctgtctcacgtgatgggctacggcttctaccacttcggcacctaccccagcggctacgagaaccctttcctgcacgccatcaacaacggcggctacaccaacacccggatcgagaagtacgaggacggcggcgtgctgcacgtgtccttcagctacagatacgaggccggcagagtgatcggcgacttcaaagtgatgggcaccggattccccgaggacagcgtgatcttcaccgacaagatcatccggtccaacgccaccgtggaacatctgcaccccatgggcgacaacgacctggacggcagcttcaccagaaccttctccctgcgggatggcggctactacagcagcgtggtggacagccacatgcacttcaagagcgccatccaccccagcatcctccagaacggcggacccatgttcgccttcagacgggtggaagaggaccacagcaacaccgagctgggcatcgtggaataccagcacgccttcaagacccccgatgccgatgccggcgaggaatgagtcgagtctagagggcccgtttaaacccgctgatcagcctcgactgtgccttctagttgccagccatctgttgtttgcccctcccccgtgccttccttgaccctggaaggtgccactcccactgtcctttcctaataaaatgaggaaattgcatcgcattgtctgagtaggtgtcattctattctggggggtggggtggggcaggacagcaagggggaggattgggaagacaatagcaggcatgctggggatgcggtgggctctatggcttctgaggcggaaagaaccagctggggctctagggggtatccccacgcgccctgtagcggcgcattaagcgcggcgggtgtggtggttacgcgcagcgtgaccgctacacttgccagcgccctagcgcccgctcctttcgctttcttcccttcctttctcgccacgttcgccggctttccccgtcaagctctaaatcgggggctccctttagggttccgatttagtgctttacggcacctcgaccccaaaaaacttgattagggtgatggttcacgtagtgggccatcgccctgatagacggtttttcgccctttgacgttggagtccacgttctttaatagtggactcttgttccaaactggaacaacactcaaccctatctcggtctattcttttgatttataagggattttgccgatttcggcctattggttaaaaaatgagctgatttaacaaaaatttaacgcgaattaattctgtggaatgtgtgtcagttagggtgtggaaagtccccaggctccccagcaggcagaagtatgcaaagcatgcatctcaattagtcagcaaccaggtgtggaaagtccccaggctccccagcaggcagaagtatgcaaagcatgcatctcaattagtcagcaaccatagtcccgcccctaactccgcccatcccgcccctaactccgcccagttccgcccattctccgccccatggctgactaattttttttatttatgcagaggccgaggccgcctctgcctctgagctattccagaagtagtgaggaggcttttttggaggcctaggcttttgcaaaaagctcccgggagcttgtatatccattttcggatctgatcaagagacaggatgaggatcgtttcgcatgattgaacaagatggattgcacgcaggttctccggccgcttgggtggagaggctattcggctatgactgggcacaacagacaatcggctgctctgatgccgccgtgttccggctgtcagcgcaggggcgcccggttctttttgtcaagaccgacctgtccggtgccctgaatgaactgcaggacgaggcagcgcggctatcgtggctggccacgacgggcgttccttgcgcagctgtgctcgacgttgtcactgaagcgggaagggactggctgctattgggcgaagtgccggggcaggatctcctgtcatctcaccttgctcctgccgagaaagtatccatcatggctgatgcaatgcggcggctgcatacgcttgatccggctacctgcccattcgaccaccaagcgaaacatcgcatcgagcgagcacgtactcggatggaagccggtcttgtcgatcaggatgatctggacgaagagcatcaggggctcgcgccagccgaactgttcgccaggctcaaggcgcgcatgcccgacggcgaggatctcgtcgtgacccatggcgatgcctgcttgccgaatatcatggtggaaaatggccgcttttctggattcatcgactgtggccggctgggtgtggcggaccgctatcaggacatagcgttggctacccgtgatattgctgaagagcttggcggcgaatgggctgaccgcttcctcgtgctttacggtatcgccgctcccgattcgcagcgcatcgccttctatcgccttcttgacgagttcttctgagcgggactctggggttcgaaatgaccgaccaagcgacgcccaacctgccatcacgagatttcgattccaccgccgccttctatgaaaggttgggcttcggaatcgttttccgggacgccggctggatgatcctccagcgcggggatctcatgctggagttcttcgcccaccccaacttgtttattgcagcttataatggttacaaataaagcaatagcatcacaaatttcacaaataaagcatttttttcactgcattctagttgtggtttgtccaaactcatcaatgtatcttatcatgtctgtataccgtcgacctctagctagagcttggcgtaatcatggtcatagctgtttcctgtgtgaaattgttatccgctcacaattccacacaacatacgagccggaagcataaagtgtaaagcctggggtgcctaatgagtgagctaactcacattaattgcgttgcgctcactgcccgctttccagtcgggaaacctgtcgtgccagctgcattaatgaatcggccaacgcgcggggagaggcggtttgcgtattgggcgctcttccgcttcctcgctcactgactcgctgcgctcggtcgttcggctgcggcgagcggtatcagctcactcaaaggcggtaatacggttatccacagaatcaggggataacgcaggaaagaacatgtgagcaaaaggccagcaaaaggccaggaaccgtaaaaaggccgcgttgctggcgtttttccataggctccgcccccctgacgagcatcacaaaaatcgacgctcaagtcagaggtggcgaaacccgacaggactataaagataccaggcgtttccccctggaagctccctcgtgcgctctcctgttccgaccctgccgcttaccggatacctgtccgcctttctcccttcgggaagcgtggcgctttctcatagctcacgctgtaggtatctcagttcggtgtaggtcgttcgctccaagctgggctgtgtgcacgaaccccccgttcagcccgaccgctgcgccttatccggtaactatcgtcttgagtccaacccggtaagacacgacttatcgccactggcagcagccactggtaacaggattagcagagcgaggtatgtaggcggtgctacagagttcttgaagtggtggcctaactacggctacactagaagaacagtatttggtatctgcgctctgctgaagccagttaccttcggaaaaagagttggtagctcttgatccggcaaacaaaccaccgctggtagcggtttttttgtttgcaagcagcagattacgcgcagaaaaaaaggatctcaagaagatcctttgatcttttctacggggtctgacgctcagtggaacgaaaactcacgttaagggattttggtcatgagattatcaaaaaggatcttcacctagatccttttaaattaaaaatgaagttttaaatcaatctaaagtatatatgagtaaacttggtctgacagttaccaatgcttaatcagtgaggcacctatctcagcgatctgtctatttcgttcatccatagttgcctgactccccgtcgtgtagataactacgatacgggagggcttaccatctggccccagtgctgcaatgataccgcgagacccacgctcaccggctccagatttatcagcaataaaccagccagccggaagggccgagcgcagaagtggtcctgcaactttatccgcctccatccagtctattaattgttgccgggaagctagagtaagtagttcgccagttaatagtttgcgcaacgttgttgccattgctacaggcatcgtggtgtcacgctcgtcgtttggtatggcttcattcagctccggttcccaacgatcaaggcgagttacatgatcccccatgttgtgcaaaaaagcggttagctccttcggtcctccgatcgttgtcagaagtaagttggccgcagtgttatcactcatggttatggcagcactgcataattctcttactgtcatgccatccgtaagatgcttttctgtgactggtgagtactcaaccaagtcattctgagaatagtgtatgcggcgaccgagttgctcttgcccggcgtcaatacgggataataccgcgccacatagcagaactttaaaagtgctcatcattggaaaacgttcttcggggcgaaaactctcaaggatcttaccgctgttgagatccagttcgatgtaacccactcgtgcacccaactgatcttcagcatcttttactttcaccagcgtttctgggtgagcaaaaacaggaaggcaaaatgccgcaaaaaagggaataagggcgacacggaaatgttgaatactcatactcttcctttttcaatattattgaagcatttatcagggttattgtctcatgagcggatacatatttgaatgtatttagaaaaataaacaaataggggttccgcgcacatttccccgaaaagtgccacctgacgtc

SEQ ID NO: 9 - DNA, 2762 bp, Artificial sequence
  AAVSI_sg-sp-opti_3 vector V2.J.6
ctaaattgtaagcgttaatattttgttaaaattcgcgttaaatttttgttaaatcagctcattttttaaccaataggccgaaatcggcaaaatcccttataaatcaaaagaatagaccgagatagggttgagtggccgctacagggcgctcccattcgccattcaggctgcgcaactgttgggaagggcgtttcggtgcgggcctcttcgctattacgccagctggcgaaagggggatgtgctgcaaggcgattaagttgggtaacgccagggttttcccagtcacgacgttgtaaaacgacggccagtgagcgcgacgtaatacgactcactatagggcgaattggcggaaggccgtcaaggccgcatggatccaaggtcgggcaggaagagggcctatttcccatgattccttcatatttgcatatacgatacaaggctgttagagagataattagaattaatttgactgtaaacacaaagatattagtacaaaatacgtgacgtagaaagtaataatttcttgggtagtttgcagttttaaaattatgttttaaaatggactatcatatgcttaccgtaacttgaaagtatttcgatttcttggctttatatatcttgtggaaaggacgaaacaccgtcaccaatcctgtccctaggtttaagagctatgctggaaacagcatagcaagtttaaataaggctagtccgttatcaacttgaaaaagtggcaccgagtcggtgctttttttcagacatccatagatctagctcgagttttttttctagactgggcctcatgggccttccgctcactgcccgctttccagtcgggaaacctgtcgtgccagctgcattaacatggtcatagctgtttccttgcgtattgggcgctctccgcttcctcgctcactgactcgctgcgctcggtcgttcgggtaaagcctggggtgcctaatgagcaaaaggccagcaaaaggccaggaaccgtaaaaaggccgcgttgctggcgtttttccataggctccgcccccctgacgagcatcacaaaaatcgacgctcaagtcagaggtggcgaaacccgacaggactataaagataccaggcgtttccccctggaagctccctcgtgcgctctcctgttccgaccctgccgcttaccggatacctgtccgcctttctcccttcgggaagcgtggcgctttctcatagctcacgctgtaggtatctcagttcggtgtaggtcgttcgctccaagctgggctgtgtgcacgaaccccccgttcagcccgaccgctgcgccttatccggtaactatcgtcttgagtccaacccggtaagacacgacttatcgccactggcagcagccactggtaacaggattagcagagcgaggtatgtaggcggtgctacagagttcttgaagtggtggcctaactacggctacactagaagaacagtatttggtatctgcgctctgctgaagccagttaccttcggaaaaagagttggtagctcttgatccggcaaacaaaccaccgctggtagcggtggtttttttgtttgcaagcagcagattacgcgcagaaaaaaaggatctcaagaagatcctttgatcttttctacggggtctgacgctcagtggaacgaaaactcacgttaagggattttggtcatgagattatcaaaaaggatcttcacctagatccttttaaattaaaaatgaagttttaaatcaatctaaagtatatatgagtaaacttggtctgacagttaccaatgcttaatcagtgaggcacctatctcagcgatctgtctatttcgttcatccatagttgcctgactccccgtcgtgtagataactacgatacgggagggcttaccatctggccccagtgctgcaatgataccgcgagaaccacgctcaccggctccagatttatcagcaataaaccagccagccggaagggccgagcgcagaagtggtcctgcaactttatccgcctccatccagtctattaattgttgccgggaagctagagtaagtagttcgccagttaatagtttgcgcaacgttgttgccattgctacaggcatcgtggtgtcacgctcgtcgtttggtatggcttcattcagctccggttcccaacgatcaaggcgagttacatgatcccccatgttgtgcaaaaaagcggttagctccttcggtcctccgatcgttgtcagaagtaagttggccgcagtgttatcactcatggttatggcagcactgcataattctcttactgtcatgccatccgtaagatgcttttctgtgactggtgagtactcaaccaagtcattctgagaatagtgtatgcggcgaccgagttgctcttgcccggcgtcaatacgggataataccgcgccacatagcagaactttaaaagtgctcatcattggaaaacgttcttcggggcgaaaactctcaaggatcttaccgctgttgagatccagttcgatgtaacccactcgtgcacccaactgatcttcagcatcttttactttcaccagcgtttctgggtgagcaaaaacaggaaggcaaaatgccgcaaaaaagggaataagggcgacacggaaatgttgaatactcatactcttcctttttcaatattattgaagcatttatcagggttattgtctcatgagcggatacatatttgaatgtatttagaaaaataaacaaataggggttccgcgcacatttccccgaaaagtgccac

SEQ ID NO: 10 - DNA, 8188 bp, Artificial sequence
gagctctactggcttctgcgccgcctctggcccactgtttccccttcccaggcaggtcctgctttctctgacctgcattctctcccctgggcctgtgccgctttctgtctgcagcttgtggcctgggtcacctctacggctggcccagatccttccctgccgcctccttcaggttccgtcttcctccactccctcttccccttgctctctgctgtgttgctgcccaaggatgctctttccggagcacttccttctcggcgctgcaccacgtgatgtcctctgagcggatcctccccgtgtctgggtcctctccgggcatctctcctccctcacccaaccccatgccgtcttcactcgctgggttcccttttccttctccttctggggcctgtgccatctctcgtttcttaggatggccttctccgacggatgtctcccttgcgtcccgcctccccttcttgtaggcctgcatcatcaccgtttttctggacaaccccaaagtaccccgtctccctggctttagccacctctccatcctcttgctttctttgcctggacaccccgttctcctgtggattcgggtcacctctcactcctttcatttgggcagctcccctaccccccttacctctctagtctgtgctagctcttccagccccctgtcatggcatcttccaggggtccgagagctcagctagtcttcttcctccaacccgggcccctatgtccacttcaggacagcatgtttgctgcctccagggatcctgtgtccccgagctgggaccaccttatattcccagggccggttaatgtggctctggttctgggtacttttatctgtcccctccaccgggtggctccggtgcccgtcagtgggcagagcgcacatcgcccacagtccccgagaagttggggggaggggtcggcaattgaaccggtgcctagagaaggtggcgcggggtaaactgggaaagtgatgtcgtgtactggctccgcctttttcccgagggtgggggagaaccgtatataagtgcagtagtcgccgtgaacgttctttttcgcaacgggtttgccgccagaacacaggtaagtgccgtgtgtggttcccgcgggcctggcctctttacgggttatggcccttgcgtgccttgaattacttccactggctgcagtacgtgattcttgatcccgagcttcgggttggaagtgggtgggagagttcgaggccttgcgcttaaggagccccttcgcctcgtgcttgagttgaggcctggcctgggcgctggggccgccgcgtgcgaatctggtggcaccttcgcgcctgtctcgctgctttcgataagtctctagccatttaaaatttttgatgacctgctgcgacgctttttttctggcaagatagtcttgtaaatgcgggccaagatctgcacactggtatttcggtttttggggccgcgggcggcgacggggcccgtgcgtcccagcgcacatgttcggcgaggcggggcctgcgagcgcggccaccgagaatcggacgggggtagtctcaagctggccggcctgctctggtgcctggcctcgcgccgccgtgtatcgccccgccctgggcggcaaggctggcccggtcggcaccagttgcgtgagcggaaagatggccgcttcccggccctgctgcagggagctcaaaatggaggacgcggcgctcgggagagcgggcgggtgagtcacccacacaaaggaaaagggcctttccgtcctcagccgtcgcttcatgtgactccacggagtaccgggcgccgtccaggcacctcgattagttctcgagcttttggagtacgtcgtctttaggttggggggaggggttttatgcgatggagtttccccacactgagtgggtggagactgaagttaggccagcttggcacttgatgtaattctccttggaatttgccctttttgagtttggatcttggttcattctcaagcctcagacagtggttcaaagtttttttcttccatttcaggtgtcgtgactgcttaagcttggtaccgccaccatggccaagggcttctacatcagcaagagcctgggcatcctgggaatcctgctgggagtggctgctgtgtgcaccatcatcgctctgagcgtggtgtacagccaggagggaggtcctggatccggaacaggtggctctggcactggaggatcaggtccaggtggatctatggtgaagcagatcgagagcaagactgctttccaggaagccttggacgctgcaggtgataagcttgtagtagttgacttctcagcaacgtggtctggaccttccaagatgatcaagcctttcttccattccctctctgagaagtattccaacgtgatattccttgaagtagatgtggatgactctcaggatgttgcttcagagtgtgaagtcaaatccatgccaacattccagttcttcaagaagggacagaaggtgggtgaattttctggagccaataaggagaagcttgaagccaccattaacgagttggtaggtaagtggctggggccagagactggctcttgaagttcctattccgaagttcctattctctagaaagtataggaacttcctggctcagaaaaagggccctgacaactcttttcatcttctaggcggttcctctacatccggtggatctggatctggagaacaaaagctcatctctgaggaggaccttggggagcagaagctaatcagtgaagaagacctcggagagcagaaattgattagcgaggaggatctttaaagacgctagcacctgatcctgatcataatcaagccatatcacatctgtagaggtttacttgctttaaaaaacctccacacctccccctgaacctgaaacataaaatgaatgcaattgttgttgttaacttgtttattgcagcttataatggttacaaataaagcaatagcatcacaaatttcacaaataaagcatttttttcactgcattctagttgtggtttgtccaaactcatcaatgtatcttatcatgtctggatctgctgaagagcgctgatcagctcttcaccatagagcccaccgcatccccagcatgcctgctattgtcttcccaatcctcccccttgctgtcctgccccaccccaccccccagaatagaatgacacctactcagacaatgcgatgcaatttcctcattttattaggaaaggacagtgggagtggcaccttccagggtcaaggaaggcacgggggaggggcaaacaacagatggctggcaactagaaggcacagtcgggtgctagctcatctgtggcccagcttgctaggcaggtcgcagtacttggccacggccatctcgtgctgttccacgtaggtttctttgtcggcctctttgatccgttccagccggtggtccacgaagtggaagccgggcatcttcaggttcttggcgggcttcttgcttctgtaggtggtcttgaaggagcagtgcaggtagcctccgcccacgagtttcagggccatctgagaatggcctctcaggccgccatcggcagggtacagcatctcggtgttggcctcccagcctctggttttcttctgcatcacggggccgttgctggggaagttcacgccgttaatcttcacgttgtagatgatgcagccgttctggaagctggtatcctgggtggcggtcagcactccgccgtcctcgtatgtggtgatccgctcccaggtgaagccctcggggaagctctgcttgaagaaatcggggatgccctgggtgtggttgatgaaggccttgctgccgtacataaagctggtggccaggatatcaaaggcgaagggcagagggccgccttccaccaccttgatcttcatggtctgggtgccctcgtaaggcttgccctcgccctcgctggtgcacttgaagtggtggttgttcacggtgccttccatgtacagcttcatgtgcatgttttctttgatcagctcgctcatggtggctacggaagttcctattccgaagttcctattcttcaaatagtataggaacttccggtaccagtcacgacacctgaaatggaagaaaaaaactttgaaccactgtctgaggcttgagaatgaaccaagatccaaactcaaaaagggcaaattccaaggagaattacatcaagtgccaagctggcctaacttcagtctccacccactcagtgtggggaaactccatcgcataaaacccctccccccaacctaaagacgacgtactccaaaagctcgagaactaatcgaggtgcctggacggcgcccggtactccgtggagtcacatgaagcgacggctgaggacggaaaggcccttttcctttgtgtgggtgactcacccgcccgctctcccgagcgccgcgtcctccattttgagctccctgcagcagggccgggaagcggccatctttccgctcacgcaactggtgccgaccgggccagccttgccgcccagggcggggcgatacacggcggcgcgaggccaggcaccagagcaggccggccagcttgagactacccccgtccgattctcggtggccgcgctcgcaggccccgcctcgccgaacatgtgcgctgggacgcacgggccccgtcgccgcccgcggccccaaaaaccgaaataccagtgtgcagatcttggcccgcatttacaagactatcttgccagaaaaaaagcgtcgcagcaggtcatcaaaaattttaaatggctagagacttatcgaaagcagcgagacaggcgcgaaggtgccaccagattcgcacgcggcggccccagcgcccaggccaggcctcaactcaagcacgaggcgaaggggctccttaagcgcaaggcctcgaactctcccacccacttccaacccgaagctcgggatcaagaatcacgtactgcagccagtggaagtaattcaaggcacgcaagggccataacccgtaaagaggccaggcccgcgggaaccacacacggcacttacctgtgttctggcggcaaacccgttgcgaaaaagaacgttcacggcgactactgcacttatatacggttctcccccaccctcgggaaaaaggcggagccagtacacgacatcactttcccagtttaccccgcgccaccttctctaggcaccggttcaattgccgacccctccccccaacttctcggggactgtgggcgatgtgcgctctgcccactgacgggcaccggagccaccggatcaggatcaggattggtgacagaaaagccccatccttaggcctcctccttcctagtctcctgatattgggtctaacccccacctcctgttaggcagattccttatctggtgacacacccccatttcctggagccatctctctccttgccagaacctctaaggtttgcttacgatggagccagagaggatcctgggagggagagcttggcagggggtgggagggaagggggggatgcgtgacctgcccggttctcagtggccaccctgcgctaccctctcccagaacctgagctgctctgacgcggctgtctggtgcgtttcactgatcctggtgctgcagcttccttacacttcccaagaggagaagcagtttggaaaaacaaaatcagaataagttggtcctgagttctaactttggctcttcacctttctagtccccaatttatattgttcctccgtgcgtcagttttacctgtgagataaggccagtagccagccccgtcctggcagggctgtggtgaggaggggggtgtccgtgtggaaaactccctttgtgagaatggtgcgtcctcgagctgggcctcatgggccttccgctcactgcccgctttccagtcgggaaacctgtcgtgccagctgcattaacatggtcatagctgtttccttgcgtattgggcgctctccgcttcctcgctcactgactcgctgcgctcggtcgttcgggtaaagcctggggtgcctaatgagcaaaaggccagcaaaaggccaggaaccgtaaaaaggccgcgttgctggcgtttttccataggctccgcccccctgacgagcatcacaaaaatcgacgctcaagtcagaggtggcgaaacccgacaggactataaagataccaggcgtttccccctggaagctccctcgtgcgctctcctgttccgaccctgccgcttaccggatacctgtccgcctttctcccttcgggaagcgtggcgctttctcatagctcacgctgtaggtatctcagttcggtgtaggtcgttcgctccaagctgggctgtgtgcacgaaccccccgttcagcccgaccgctgcgccttatccggtaactatcgtcttgagtccaacccggtaagacacgacttatcgccactggcagcagccactggtaacaggattagcagagcgaggtatgtaggcggtgctacagagttcttgaagtggtggcctaactacggctacactagaagaacagtatttggtatctgcgctctgctgaagccagttaccttcggaaaaagagttggtagctcttgatccggcaaacaaaccaccgctggtagcggtggtttttttgtttgcaagcagcagattacgcgcagaaaaaaaggatctcaagaagatcctttgatcttttctacggggtctgacgctcagtggaacgaaaactcacgttaagggattttggtcatgagattatcaaaaaggatcttcacctagatccttttaaattaaaaatgaagttttaaatcaatctaaagtatatatgagtaaacttggtctgacagttaccaatgcttaatcagtgaggcacctatctcagcgatctgtctatttcgttcatccatagttgcctgactccccgtcgtgtagataactacgatacgggagggcttaccatctggccccagtgctgcaatgataccgcgagaaccacgctcaccggctccagatttatcagcaataaaccagccagccggaagggccgagcgcagaagtggtcctgcaactttatccgcctccatccagtctattaattgttgccgggaagctagagtaagtagttcgccagttaatagtttgcgcaacgttgttgccattgctacaggcatcgtggtgtcacgctcgtcgtttggtatggcttcattcagctccggttcccaacgatcaaggcgagttacatgatcccccatgttgtgcaaaaaagcggttagctccttcggtcctccgatcgttgtcagaagtaagttggccgcagtgttatcactcatggttatggcagcactgcataattctcttactgtcatgccatccgtaagatgcttttctgtgactggtgagtactcaaccaagtcattctgagaatagtgtatgcggcgaccgagttgctcttgcccggcgtcaatacgggataataccgcgccacatagcagaactttaaaagtgctcatcattggaaaacgttcttcggggcgaaaactctcaaggatcttaccgctgttgagatccagttcgatgtaacccactcgtgcacccaactgatcttcagcatcttttactttcaccagcgtttctgggtgagcaaaaacaggaaggcaaaatgccgcaaaaaagggaataagggcgacacggaaatgttgaatactcatactcttcctttttcaatattattgaagcatttatcagggttattgtctcatgagcggatacatatttgaatgtatttagaaaaataaacaaataggggttccgcgcacatttccccgaaaagtgccacctaaattgtaagcgttaatattttgttaaaattcgcgttaaatttttgttaaatcagctcattttttaaccaataggccgaaatcggcaaaatcccttataaatcaaaagaatagaccgagatagggttgagtggccgctacagggcgctcccattcgccattcaggctgcgcaactgttgggaagggcgtttcggtgcgggcctcttcgctattacgccagctggcgaaagggggatgtgctgcaaggcgattaagttgggtaacgccagggttttcccagtcacgacgttgtaaaacgacggccagtgagcgcgacgtaatacgactcactatagggcgaattggcggaaggccgtcaaggccgcatgaatt

SEQ ID NO: 11 - DNA, 3996 bp, Artificial sequence
  M2-gene-Long_RSV1-FLAG_Tx V12.A.8
gaagttcctattccgaagttcctattctctagaaagtataggaacttcctggctcagaaaaagggccctgacaactcttttcatcttctaggcggttcctctacatccggtggatctggatctgggcatgtggttgaggggcttgctggcgaactagagcaattgcgagcccgcctcgaacaccatcctcaaggtcaataaagactcgagcacctgatcctgatcataatcaagccatatcacatctgtagaggtttacttgctttaaaaaacctccacacctccccctgaacctgaaacataaaatgaatgcaattgttgttgttaacttgtttattgcagcttataatggttacaaataaagcaatagcatcacaaatttcacaaataaagcatttttttcactgcattctagttgtggtttgtccaaactcatcaatgtatcttatcatgtctggatctgctgaagagcgctgatcagctcttcaccatagagcccaccgcatccccagcatgcctgctattgtcttcccaatcctcccccttgctgtcctgccccaccccaccccccagaatagaatgacacctactcagacaatgcgatgcaatttcctcattttattaggaaaggacagtgggagtggcaccttccagggtcaaggaaggcacgggggaggggcaaacaacagatggctggcaactagaaggcacagtcgggtgctagcgaagaccgagcggtggatccgtatggtgacaagacgactagtgtgaacgacctgttagagaacccggcacatctgtcgagaggtacgaccgtgcactaagcttcgcaaggtcagtggagctatcgagtgtaggatggttcaagtctgccaatggagctacagaagtcgaagccgtccagatctggactatagtcacttatcgtcatcgtccttataatcaatatcgtggtctttataatctccatcatgatccttgtaatccccgggggtggtatcgttgttcttggcgtggtcgttggtgtcgttgacggtgctctctttgggattgttgatggtgatgctcttgtggatgtccagggtgttcttgatggttttcttcagcacgtcggcaggcagccgcttcagcagatggatggtctgcttgttgttcttccggttgctctcgatgtagctgatcacggtgttgtacacccggatcttggggctgttaggttcctcgttgtcccgcagcttcttgatgtcgtcgctgttcagctctgtcagcagcttgctcatggccacgcaggcgctctgcttggtgatgttgttgatgctgccgatatagctttccagcacgcccacaacgcccagggcatattcctcggttctatccagttcggcggctccgctgatctcgctcagggtgtcgatgctcttatccatggacttcaggattctgttcagcatgaagttctgccgcacgagcagagcgtgaggaggccactcgaagtagttgtggctgaagtggcatctcttgccgttcaggcagtggcctctgatctcgaacttgcaggggttccgtctgctcatggtggcggtattgtcttcggtaccgcacgaagttcctattcggaagttcctattcttcaaatagtataggaacttccgctctgaccagctgcattaacatggtcatagctgtttccttgcgtattgggcgctctccgcttcctcgctcactgactcgctgcgctcggtcgttcgggtaaagcctggggtgcctaatgagcaaaaggccagcaaaaggccaggaaccgtaaaaaggccgcgttgctggcgtttttccataggctccgcccccctgacgagcatcacaaaaatcgacgctcaagtcagaggtggcgaaacccgacaggactataaagataccaggcgtttccccctggaagctccctcgtgcgctctcctgttccgaccctgccgcttaccggatacctgtccgcctttctcccttcgggaagcgtggcgctttctcatagctcacgctgtaggtatctcagttcggtgtaggtcgttcgctccaagctgggctgtgtgcacgaaccccccgttcagcccgaccgctgcgccttatccggtaactatcgtcttgagtccaacccggtaagacacgacttatcgccactggcagcagccactggtaacaggattagcagagcgaggtatgtaggcggtgctacagagttcttgaagtggtggcctaactacggctacactagaagaacagtatttggtatctgcgctctgctgaagccagttaccttcggaaaaagagttggtagctcttgatccggcaaacaaaccaccgctggtagcggtggtttttttgtttgcaagcagcagattacgcgcagaaaaaaaggatctcaagaagatcctttgatcttttctacggggtctgacgctcagtggaacgaaaactcacgttaagggattttggtcatgagattatcaaaaaggatcttcacctagatccttttaaattaaaaatgaagttttaaatcaatctaaagtatatatgagtaaacttggtctgacagttaccaatgcttaatcagtgaggcacctatctcagcgatctgtctatttcgttcatccatagttgcctgactccccgtcgtgtagataactacgatacgggagggcttaccatctggccccagtgctgcaatgataccgcgagaaccacgctcaccggctccagatttatcagcaataaaccagccagccggaagggccgagcgcagaagtggtcctgcaactttatccgcctccatccagtctattaattgttgccgggaagctagagtaagtagttcgccagttaatagtttgcgcaacgttgttgccattgctacaggcatcgtggtgtcacgctcgtcgtttggtatggcttcattcagctccggttcccaacgatcaaggcgagttacatgatcccccatgttgtgcaaaaaagcggttagctccttcggtcctccgatcgttgtcagaagtaagttggccgcagtgttatcactcatggttatggcagcactgcataattctcttactgtcatgccatccgtaagatgcttttctgtgactggtgagtactcaaccaagtcattctgagaatagtgtatgcggcgaccgagttgctcttgcccggcgtcaatacgggataataccgcgccacatagcagaactttaaaagtgctcatcattggaaaacgttcttcggggcgaaaactctcaaggatcttaccgctgttgagatccagttcgatgtaacccactcgtgcacccaactgatcttcagcatcttttactttcaccagcgtttctgggtgagcaaaaacaggaaggcaaaatgccgcaaaaaagggaataagggcgacacggaaatgttgaatactcatactcttcctttttcaatattattgaagcatttatcagggttattgtctcatgagcggatacatatttgaatgtatttagaaaaataaacaaataggggttccgcgcacatttccccgaaaagtgccacctaaattgtaagcgttaatattttgttaaaattcgcgttaaatttttgttaaatcagctcattttttaaccaataggccgaaatcggcaaaatcccttataaatcaaaagaatagaccgagatagggttgagtggccgctacagggcgctcccattcgccattcaggctgcgcaactgttgggaagggcgtttcggtgcgggcctcttcgctattacgccagctggcgaaagggggatgtgctgcaaggcgattaagttgggtaacgccagggttttcccagtcacgacgttgtaaaacgacggccagtgagcgcgacgtaatacgactcactatagggcgaattggcggaaggccgtcaaggccgcatgaattcgctaccgggagttggtaggtaagtggctggggccagagactggctctt

SEQ ID NO: 12 - DNA, 20 bp, Artificial sequence
  turboRFP_GT_F1 1.I.7
gagaggccattctcagatgg

SEQ ID NO: 13 - DNA, 20 bp, Artificial sequence
  turboRFP_GT_R1 1.I.8
cgggcatcttcaggttcttg

SEQ ID NO: 14 - DNA, 25 bp, Artificial sequence
  turboRFP_probe_FAM 1.I.9
ctacctgcactgctccttcaagacc

SEQ ID NO: 15 - DNA, 26 bp, Artificial sequence
  TRAC_TCRA-promoter_F1 10.A.10
gacttgtcactggatttagagtctct

SEQ ID NO: 16 - DNA, 22 bp, Artificial sequence
  TRAC_probe (HEX) 10.B.6
atccagaaccctgaccctgccg

SEQ ID NO: 17 - DNA, 23 bp, Artificial sequence
  TRAC-TCRA-ex1-F1 10.A.9
ctgatcctcttgtcccacagata

SEQ ID NO: 18 - DNA, 19 bp, Artificial sequence
  AAVS1_GT_F5 15.F.9
actctgccctctaacgctg

SEQ ID NO: 19 - DNA, 20 bp, Artificial sequence
  AMPN-TMD_GT_R1 19.E.7
gctgatgtagaagcccttgg

SEQ ID NO: 20 - DNA, 876 bp, Artificial sequence
  SurfaceTag with Barcode FLAG-MYC-HA
atggaggagggacagtacagcgagatcgaggagctgcccaggagaaggtgctgcaggagaggcacccagatcgtgctgctgggactggtgaccgctgctctgtgggcaggactgctgacattgctgttgctgtggcactgggacaccacccagagcctgaagcagctggaggagggaggtcctggatccggaacaggtggctctggcactggaggatcaggtccaggtggatctatggtgaagcagatcgagagcaagactgctttccaggaagccttggacgctgcaggtgataagcttgtagtagttgacttctcagcaacgtggtctggaccttccaagatgatcaagcctttcttccattccctctctgagaagtattccaacgtgatattccttgaagtagatgtggatgactctcaggatgttgcttcagagtgtgaagtcaaatccatgccaacattccagttcttcaagaagggacagaaggtgggtgaattttctggagccaataaggagaagcttgaagccaccattaacgagttggtcggtggttcctctacatccggtggatctggatctggtgattacaaggatcatgatggagattataaagaccacgatattgattataaggacgatgacgataagggaggatatccgtatgatgtaccagactacgctggatacccttacgatgtacctgattatgccggatacccctatgacgtaccggactatgcgggaggagaacaaaagctcatctctgaggaggaccttggggagcagaagctaatcagtgaagaggacctcggagagcagaaattgattagcgaagaggatcttggcgggcaccatcatcatcaccaccactaa

SEQ ID NO: 21 - DNA, 20 bp, Artificial sequence
  ORF-AM_GT_F2
ttctgtagctccattggcag

SEQ ID NO: 22 - DNA, 20 bp, Artificial sequence
  ORF-AM_GT_R1
atccgtatggtgacaagacg

SEQ ID NO: 23 - DNA, 26 bp, Artificial sequence
  TRAC-TCRA-ex1-F1
gacttgtcactggatttagagtctct